European Patent Specification EP 3 897 693 B1, published August 6, 2025. Title: Synthetische und rekombinant hergestellte Kollagenpeptide mit biologischer Wirksamkeit. Applicant: GELITA AG. The sequence listing filed with the application follows.

SEQUENCE LISTING (30 sequences)

SEQ ID NO: 1 - protein, 11 aa, Artificial Sequence
  Artificial collagen sequence
LTGPIGPPGPA

SEQ ID NO: 2 - protein, 33 aa, Artificial Sequence
  Artificial collagen sequence
GAPGKDGVRGLTGPIGPPGPAGAPGDKGEAGPS

SEQ ID NO: 3 - protein, 24 aa, Artificial Sequence
  Artificial collagen sequence
GAPGKDGVRGLTGPIGPPGPAGAP

SEQ ID NO: 4 - protein, 24 aa, Artificial Sequence
  Artificial collagen sequence
GAPGKDGVRGLTGPIGPPGPAGAR

SEQ ID NO: 5 - protein, 24 aa, Artificial Sequence
  Artificial collagen sequence
GRPGPPGPPGARGQAGVMGFPGPK

SEQ ID NO: 6 - protein, 11 aa, Artificial Sequence
  Artificial collagen sequence
  MOD_RES (8)..(8): 4Hyp
LTGPIGPPGPA

SEQ ID NO: 7 - protein, 33 aa, Artificial Sequence; identical to SEQ ID NO: 2
  Artificial collagen sequence
  MOD_RES (3)..(3): 4Hyp
  MOD_RES (18)..(18): 4Hyp
  MOD_RES (24)..(24): 4Hyp

SEQ ID NO: 8 - protein, 24 aa, Artificial Sequence
  Artificial collagen sequence
  MOD_RES (3)..(3): 4Hyp
  MOD_RES (18)..(18): 4Hyp
  MOD_RES (24)..(24): 4Hyp
GAPGKDGVRGLTGPIGPPGPAGAP

SEQ ID NO: 9 - protein, 24 aa, Artificial Sequence
  Artificial collagen sequence
  MOD_RES (3)..(3): 4Hyp
  MOD_RES (18)..(18): 4Hyp
GAPGKDGVRGLTGPIGPPGPAGAR

SEQ ID NO: 10 - protein, 24 aa, Artificial Sequence
  Artificial collagen sequence
  MOD_RES (3)..(3): 4Hyp
  MOD_RES (9)..(9): 4Hyp
  MOD_RES (21)..(21): 4Hyp
GRPGPPGPPGARGQAGVMGFPGPK

SEQ ID NO: 11 - protein, 11 aa, Artificial Sequence
  Artificial collagen sequence
GAPGKDGVRGL

SEQ ID NO: 12 - protein, 23 aa, Artificial Sequence
  Artificial collagen sequence
GAPGKDGVRGLTGPIGPPGPAGA

SEQ ID NO: 13 - protein, 58 aa, Artificial Sequence
  Artificial collagen sequence
GAPGKDGVRGLTGPIGPPGPAGAPGDKGEAGPSGPAGPTGARGAPGDRGEPGPPGPAG

SEQ ID NO: 14 - protein, 90 aa, Artificial Sequence
  Artificial collagen sequence
GAPGKDGVRGLTGPIGPPGPAGAPGDKGEAGPSGPAGPTGARGAPGDRGEPGPPGPAGFAGPPGADGQPGAKGEPGDAGAKGDAGPPGPA

SEQ ID NO: 15 - protein, 19 aa, Artificial Sequence
  Artificial collagen sequence
KGAPGADGPAGAPGTPGPQ

SEQ ID NO: 16 - protein, 35 aa, Artificial Sequence
  Artificial collagen sequence
GPPGPAGEKGAPGADGPAGAPGTPGPQGIAGQRGV

SEQ ID NO: 17 - protein, 11 aa, Artificial Sequence
  Artificial collagen sequence
  MOD_RES (3)..(3): 4Hyp
GAPGKDGVRGL

SEQ ID NO: 18 - protein, 23 aa, Artificial Sequence
  Artificial collagen sequence
  MOD_RES (3)..(3): 4Hyp
  MOD_RES (18)..(18): 4Hyp
GAPGKDGVRGLTGPIGPPGPAGA

SEQ ID NO: 19 - protein, 58 aa, Artificial Sequence; identical to SEQ ID NO: 13
  Artificial collagen sequence
  MOD_RES (3)..(3): 4Hyp
  MOD_RES (18)..(18): 4Hyp
  MOD_RES (24)..(24): 4Hyp
  MOD_RES (45)..(45): 4Hyp
  MOD_RES (51)..(51): 4Hyp
  MOD_RES (54)..(54): 4Hyp

SEQ ID NO: 20 - protein, 90 aa, Artificial Sequence; identical to SEQ ID NO: 14
  Artificial collagen sequence
  MOD_RES (3)..(3): 4Hyp
  MOD_RES (18)..(18): 4Hyp
  MOD_RES (24)..(24): 4Hyp
  MOD_RES (45)..(45): 4Hyp
  MOD_RES (51)..(51): 4Hyp
  MOD_RES (54)..(54): 4Hyp
  MOD_RES (63)..(63): 4Hyp
  MOD_RES (69)..(69): 4Hyp

SEQ ID NO: 21 - protein, 19 aa, Artificial Sequence
  Artificial collagen sequence
  MOD_RES (4)..(4): 4Hyp
  MOD_RES (13)..(13): 4Hyp
KGAPGADGPAGAPGTPGPQ

SEQ ID NO: 22 - protein, 35 aa, Artificial Sequence; identical to SEQ ID NO: 16
  Artificial collagen sequence
  MOD_RES (3)..(3): 4Hyp
  MOD_RES (12)..(12): 4Hyp
  MOD_RES (21)..(21): 4Hyp

SEQ ID NO: 23 - protein, 33 aa, Artificial Sequence
  Artificial collagen sequence
  MOD_RES (3)..(3): 4Hyp
  MOD_RES (18)..(18): 4Hyp
  MOD_RES (24)..(24): 4Hyp
GVPGKYGVRGLTGPIGPPGPLGIPGWKGFVGPT

SEQ ID NO: 24 - protein, 36 aa, Artificial Sequence
  Artificial collagen sequence
  MOD_RES (3)..(3): 4Hyp
  MOD_RES (12)..(12): 4Hyp
  MOD_RES (21)..(21): 4Hyp
GPPGPVGTKGIPGVYGPLGIPGTPGPWGILGTKRGV

SEQ ID NO: 25 - protein, 33 aa, Artificial Sequence; identical to SEQ ID NO: 2
  Artificial collagen sequence
  MOD_RES (3)..(3): 4Hyp
  MOD_RES (14)..(14): 4Hyp
  MOD_RES (17)..(17): 4Hyp
  MOD_RES (18)..(18): 4Hyp
  MOD_RES (20)..(20): 4Hyp
  MOD_RES (24)..(24): 4Hyp
  MOD_RES (32)..(32): 4Hyp

SEQ ID NO: 26 - protein, 39 aa, Artificial Sequence
  Artificial collagen sequence
  MOD_RES (9)..(9): 4Hyp
  MOD_RES (24)..(24): 4Hyp
  MOD_RES (30)..(30): 4Hyp
HHHHHHGAPGKDGVRGLTGPIGPPGPAGAPGDKGEAGPS

SEQ ID NO: 27 - protein, 33 aa, Artificial Sequence
  Artificial collagen sequence
  MOD_RES (3)..(3): 4Hyp
  MOD_RES (18)..(18): 4Hyp
  MOD_RES (24)..(24): 4Hyp
GLPGKMGVFGLTGPIGPPGPWGVPGHKGYLGPT

SEQ ID NO: 28 - protein, 33 aa, Artificial Sequence
  Artificial collagen sequence
  MOD_RES (3)..(3): 4Hyp
  MOD_RES (18)..(18): 4Hyp
  MOD_RES (24)..(24): 4Hyp
GLPGKYGVHGLTGPLGPPGPMGIPGWKGFVGPT

SEQ ID NO: 29 - protein, 35 aa, Artificial Sequence
  Artificial collagen sequence
  MOD_RES (3)..(3): 4Hyp
  MOD_RES (12)..(12): 4Hyp
  MOD_RES (21)..(21): 4Hyp
GPPGPLGMKGLPGVWGPFGLPGTPGPHGITGYKGV

SEQ ID NO: 30 - protein, 35 aa, Artificial Sequence
  Artificial collagen sequence
  MOD_RES (3)..(3): 4Hyp
  MOD_RES (12)..(12): 4Hyp
  MOD_RES (21)..(21): 4Hyp
GPPGPVGTKGLPGFYGPLGIPGHPGPWGMLGTKGV